European Patent Application EP 4 289 939 A1, published December 13, 2023. Title: Population of transfected immune cells and method for their production. Applicant: Apeiron Biologics AG invIOs GmbH. The sequence listing filed with the application follows.

SEQUENCE LISTING (68 sequences)

SEQ ID NO: 1 - RNA, 21 nt, Artificial Sequence
  siRNA
  modified_base 20: /mod_base="OTHER" /note="deoxy-thymidine"
  modified_base 21: /mod_base="OTHER" /note="deoxy-thymidine"
gugagaaugaguacuuuaann

SEQ ID NO: 2 - RNA, 21 nt, Artificial Sequence
  siRNA
  modified_base 20: /mod_base="OTHER" /note="deoxy-thymidine"
  modified_base 21: /mod_base="OTHER" /note="deoxy-thymidine"
uuaaaguacucauucucacnn

SEQ ID NO: 3 - RNA, 21 nt, Artificial Sequence
  siRNA
  modified_base 1: /mod_base="gm"
  modified_base 3: /mod_base="gm"
  modified_base 18: /mod_base="OTHER" /note="2'-O-methyl-adenosine"
  modified_base 20: /mod_base="OTHER" /note="deoxy-thymidine"
  modified_base 21: /mod_base="OTHER" /note="deoxy-thymidine"
gugagaaugaguacuuuaann

SEQ ID NO: 4 - RNA, 21 nt, Artificial Sequence
  siRNA
  modified_base 3: /mod_base="OTHER" /note="2'-O-methyl-adenosine"
  modified_base 17: /mod_base="cm"
  modified_base 19: /mod_base="cm"
  modified_base 20: /mod_base="OTHER" /note="deoxy-thymidine"
  modified_base 21: /mod_base="OTHER" /note="deoxy-thymidine"
uuaaaguacucauucucacnn

SEQ ID NO: 5 - RNA, 21 nt, Artificial Sequence
  siRNA
  modified_base 1: /mod_base="gm"
  modified_base 3: /mod_base="gm"
  modified_base 20: /mod_base="OTHER" /note="deoxy-thymidine"
  modified_base 21: /mod_base="OTHER" /note="deoxy-thymidine"
gugagaaugaguacuuuaann

SEQ ID NO: 6 - RNA, 21 nt, Artificial Sequence
  siRNA
  modified_base 1: /mod_base="um"
  modified_base 2: /mod_base="um"
  modified_base 20: /mod_base="OTHER" /note="deoxy-thymidine"
  modified_base 21: /mod_base="OTHER" /note="deoxy-thymidine"
nnaaaguacucauucucacnn

SEQ ID NO: 7 - RNA, 21 nt, Artificial Sequence
  siRNA
  modified_base 1: /mod_base="gm"
  modified_base 3: /mod_base="gm"
  modified_base 20: /mod_base="OTHER" /note="deoxy-thymidine"
  modified_base 21: /mod_base="OTHER" /note="deoxy-thymidine"
gugagaaugaguacuuuaann

SEQ ID NO: 8 - RNA, 21 nt, Artificial Sequence
  siRNA
  modified_base 2: /mod_base="um"
  modified_base 20: /mod_base="OTHER" /note="deoxy-thymidine"
  modified_base 21: /mod_base="OTHER" /note="deoxy-thymidine"
unaaaguacucauucucacnn

SEQ ID NO: 9 - RNA, 21 nt, Artificial Sequence
  siRNA
  modified_base 1: /mod_base="gm"
  modified_base 3: /mod_base="gm"
  modified_base 18: /mod_base="OTHER" /note="2'-O-methyl-adenosine"
  modified_base 20: /mod_base="OTHER" /note="deoxy-thymidine"
  modified_base 21: /mod_base="OTHER" /note="deoxy-thymidine"
gugagaaugaguacuuuaann

SEQ ID NO: 10 - RNA, 21 nt, Artificial Sequence
  siRNA
  modified_base 2: /mod_base="um"
  modified_base 20: /mod_base="OTHER" /note="deoxy-thymidine"
  modified_base 21: /mod_base="OTHER" /note="deoxy-thymidine"
unaaaguacucauucucacnn

SEQ ID NO: 11 - RNA, 21 nt, Artificial Sequence
  siRNA
  modified_base 1: /mod_base="gm"
  modified_base 3: /mod_base="gm"
  modified_base 18: /mod_base="OTHER" /note="2'-O-methyl-adenosine"
  modified_base 19: /mod_base="OTHER" /note="2'-O-methyl-adenosine"
  modified_base 20: /mod_base="OTHER" /note="deoxy-thymidine"
  modified_base 21: /mod_base="OTHER" /note="deoxy-thymidine"
gugagaaugaguacuuuaann

SEQ ID NO: 12 - RNA, 21 nt, Artificial Sequence
  siRNA
  modified_base 1: /mod_base="um"
  modified_base 2: /mod_base="um"
  modified_base 20: /mod_base="OTHER" /note="deoxy-thymidine"
  modified_base 21: /mod_base="OTHER" /note="deoxy-thymidine"
nnaaaguacucauucucacnn

SEQ ID NO: 13 - RNA, 21 nt, Artificial Sequence
  siRNA
  modified_base 15: /mod_base="um"
  modified_base 16: /mod_base="um"
  modified_base 18: /mod_base="OTHER" /note="2'-O-methyl-adenosine"
  modified_base 20: /mod_base="OTHER" /note="deoxy-thymidine"
  modified_base 21: /mod_base="OTHER" /note="deoxy-thymidine"
gugagaaugaguacnnuaann

SEQ ID NO: 14 - RNA, 21 nt, Artificial Sequence
  siRNA
  modified_base 2: /mod_base="um"
  modified_base 20: /mod_base="OTHER" /note="deoxy-thymidine"
  modified_base 21: /mod_base="OTHER" /note="deoxy-thymidine"
unaaaguacucauucucacnn

SEQ ID NO: 15 - RNA, 21 nt, Artificial Sequence
  siRNA
  modified_base 15: /mod_base="um"
  modified_base 16: /mod_base="um"
  modified_base 18: /mod_base="OTHER" /note="2'-O-methyl-adenosine"
  modified_base 19: /mod_base="OTHER" /note="2'-O-methyl-adenosine"
  modified_base 20: /mod_base="OTHER" /note="deoxy-thymidine"
  modified_base 21: /mod_base="OTHER" /note="deoxy-thymidine"
gugagaaugaguacnnuaann

SEQ ID NO: 16 - RNA, 21 nt, Artificial Sequence
  siRNA
  modified_base 1: /mod_base="um"
  modified_base 2: /mod_base="um"
  modified_base 20: /mod_base="OTHER" /note="deoxy-thymidine"
  modified_base 21: /mod_base="OTHER" /note="deoxy-thymidine"
nnaaaguacucauucucacnn

SEQ ID NO: 17 - RNA, 21 nt, Artificial Sequence
  siRNA
  modified_base 2: /mod_base="um"
  modified_base 4: /mod_base="OTHER" /note="2'-O-methyl-adenosine"
  modified_base 6: /mod_base="OTHER" /note="2'-O-methyl-adenosine"
  modified_base 8: /mod_base="um"
  modified_base 10: /mod_base="OTHER" /note="2'-O-methyl-adenosine"
  modified_base 12: /mod_base="um"
  modified_base 14: /mod_base="cm"
  modified_base 16: /mod_base="um"
  modified_base 18: /mod_base="OTHER" /note="2'-O-methyl-adenosine"
  modified_base 20: /mod_base="OTHER" /note="deoxy-thymidine"
  modified_base 21: /mod_base="OTHER" /note="deoxy-thymidine"
gngagaangagnacunuaann

SEQ ID NO: 18 - RNA, 21 nt, Artificial Sequence
  siRNA
  modified_base 20: /mod_base="OTHER" /note="deoxy-thymidine"
  modified_base 21: /mod_base="OTHER" /note="deoxy-thymidine"
uuaaaguacucauucucacnn

SEQ ID NO: 19 - RNA, 21 nt, Artificial Sequence
  siRNA
  modified_base 20: /mod_base="OTHER" /note="deoxy-thymidine"
  modified_base 21: /mod_base="OTHER" /note="deoxy-thymidine"
gugagaaugaguacuuuaann

SEQ ID NO: 20 - RNA, 21 nt, Artificial Sequence
  siRNA
  modified_base 1: /mod_base="um"
  modified_base 3: /mod_base="OTHER" /note="2'-O-methyl-adenosine"
  modified_base 5: /mod_base="OTHER" /note="2'-O-methyl-adenosine"
  modified_base 7: /mod_base="um"
  modified_base 9: /mod_base="cm"
  modified_base 11: /mod_base="cm"
  modified_base 13: /mod_base="um"
  modified_base 15: /mod_base="cm"
  modified_base 17: /mod_base="cm"
  modified_base 19: /mod_base="cm"
  modified_base 20: /mod_base="OTHER" /note="deoxy-thymidine"
  modified_base 21: /mod_base="OTHER" /note="deoxy-thymidine"
nuaaagnacucanucucacnn

SEQ ID NO: 21 - RNA, 21 nt, Artificial Sequence
  siRNA
  modified_base 1: /mod_base="gm"
  modified_base 3: /mod_base="gm"
  modified_base 5: /mod_base="gm"
  modified_base 18: /mod_base="OTHER" /note="2'-O-methyl-adenosine"
  modified_base 20: /mod_base="OTHER" /note="deoxy-thymidine"
  modified_base 21: /mod_base="OTHER" /note="deoxy-thymidine"
gugagaaugaguacuuuaann

SEQ ID NO: 22 - RNA, 21 nt, Artificial Sequence
  siRNA
  modified_base 3: /mod_base="OTHER" /note="2'-O-methyl-adenosine"
  modified_base 15: /mod_base="cm"
  modified_base 17: /mod_base="cm"
  modified_base 19: /mod_base="cm"
  modified_base 20: /mod_base="OTHER" /note="deoxy-thymidine"
  modified_base 21: /mod_base="OTHER" /note="deoxy-thymidine"
uuaaaguacucauucucacnn

SEQ ID NO: 23 - RNA, 21 nt, Artificial Sequence
  siRNA
  modified_base 20: /mod_base="OTHER" /note="deoxy-thymidine"
  modified_base 21: /mod_base="OTHER" /note="deoxy-thymidine"
gugagaaugaguacuuuaann

SEQ ID NO: 24 - RNA, 21 nt, Artificial Sequence
  siRNA
  modified_base 1: /mod_base="OTHER" /note="2'-fluoro deoxyuridine"
  modified_base 2: /mod_base="OTHER" /note="2'-fluoro deoxyuridine"
  modified_base 7: /mod_base="OTHER" /note="2'-fluoro deoxyuridine"
  modified_base 9: /mod_base="OTHER" /note="2'-fluoro deoxycytosine"
  modified_base 10: /mod_base="OTHER" /note="2'-fluoro deoxyuridine"
  modified_base 11: /mod_base="OTHER" /note="2'-fluoro deoxycytosine"
  modified_base 13: /mod_base="OTHER" /note="2'-fluoro deoxyuridine"
  modified_base 14: /mod_base="OTHER" /note="2'-fluoro deoxyuridine"
  modified_base 15: /mod_base="OTHER" /note="2'-fluoro deoxycytosine"
  modified_base 16: /mod_base="OTHER" /note="2'-fluoro deoxyuridine"
  modified_base 17: /mod_base="OTHER" /note="2'-fluoro deoxycytosine"
  modified_base 19: /mod_base="OTHER" /note="2'-fluoro deoxycytosine"
  modified_base 20: /mod_base="OTHER" /note="deoxy-thymidine"
  modified_base 21: /mod_base="OTHER" /note="deoxy-thymidine"
nnaaagnacncanncncacnn

SEQ ID NO: 25 - RNA, 21 nt, Artificial Sequence
  siRNA
  modified_base 2: /mod_base="OTHER" /note="2'-fluoro deoxyuridine"
  modified_base 8: /mod_base="OTHER" /note="2'-fluoro deoxyuridine"
  modified_base 12: /mod_base="OTHER" /note="2'-fluoro deoxyuridine"
  modified_base 14: /mod_base="OTHER" /note="2'-fluoro deoxycytosine"
  modified_base 15: /mod_base="OTHER" /note="2'-fluoro deoxyuridine"
  modified_base 16: /mod_base="OTHER" /note="2'-fluoro deoxyuridine"
  modified_base 17: /mod_base="OTHER" /note="2'-fluoro deoxyuridine"
  modified_base 20: /mod_base="OTHER" /note="deoxy-thymidine"
  modified_base 21: /mod_base="OTHER" /note="deoxy-thymidine"
gngagaangagnacnnnaann

SEQ ID NO: 26 - RNA, 21 nt, Artificial Sequence
  siRNA
  modified_base 20: /mod_base="OTHER" /note="deoxy-thymidine"
  modified_base 21: /mod_base="OTHER" /note="deoxy-thymidine"
uuaaaguacucauucucacnn

SEQ ID NO: 27 - RNA, 21 nt, Artificial Sequence
  siRNA
  modified_base 4: /mod_base="OTHER" /note="2'-O-methyl-adenosine"
  modified_base 7: /mod_base="OTHER" /note="2'-O-methyl-adenosine"
  modified_base 10: /mod_base="OTHER" /note="2'-O-methyl-adenosine"
  modified_base 20: /mod_base="OTHER" /note="deoxy-thymidine"
  modified_base 21: /mod_base="OTHER" /note="deoxy-thymidine"
gugagaaugaguacuuuaann

SEQ ID NO: 28 - RNA, 21 nt, Artificial Sequence
  siRNA
  modified_base 1: /mod_base="OTHER" /note="2'-fluoro deoxyuridine"
  modified_base 2: /mod_base="OTHER" /note="2'-fluoro deoxyuridine"
  modified_base 7: /mod_base="OTHER" /note="2'-fluoro deoxyuridine"
  modified_base 9: /mod_base="OTHER" /note="2'-fluoro deoxycytosine"
  modified_base 10: /mod_base="OTHER" /note="2'-fluoro deoxyuridine"
  modified_base 11: /mod_base="OTHER" /note="2'-fluoro deoxycytosine"
  modified_base 13: /mod_base="OTHER" /note="2'-fluoro deoxyuridine"
  modified_base 14: /mod_base="OTHER" /note="2'-fluoro deoxyuridine"
  modified_base 15: /mod_base="OTHER" /note="2'-fluoro deoxycytosine"
  modified_base 16: /mod_base="OTHER" /note="2'-fluoro deoxyuridine"
  modified_base 17: /mod_base="OTHER" /note="2'-fluoro deoxycytosine"
  modified_base 19: /mod_base="OTHER" /note="2'-fluoro deoxycytosine"
  modified_base 20: /mod_base="OTHER" /note="deoxy-thymidine"
  modified_base 21: /mod_base="OTHER" /note="deoxy-thymidine"
nnaaagnacncanncncacnn

SEQ ID NO: 29 - RNA, 21 nt, Artificial Sequence
  siRNA
  modified_base 1: /mod_base="gm"
  modified_base 3: /mod_base="gm"
  modified_base 20: /mod_base="OTHER" /note="deoxy-thymidine"
  modified_base 21: /mod_base="OTHER" /note="deoxy-thymidine"
gugagaaugaguacuuuaann

SEQ ID NO: 30 - RNA, 21 nt, Artificial Sequence
  siRNA
  modified_base 13: /mod_base="OTHER" /note="2'-fluoro deoxyuridine"
  modified_base 14: /mod_base="OTHER" /note="2'-fluoro deoxyuridine"
  modified_base 15: /mod_base="OTHER" /note="2'-fluoro deoxycytosine"
  modified_base 16: /mod_base="OTHER" /note="2'-fluoro deoxyuridine"
  modified_base 17: /mod_base="OTHER" /note="2'-fluoro deoxycytosine"
  modified_base 19: /mod_base="OTHER" /note="2'-fluoro deoxycytosine"
  modified_base 20: /mod_base="OTHER" /note="deoxy-thymidine"
  modified_base 21: /mod_base="OTHER" /note="deoxy-thymidine"
uuaaaguacucanncncacnn

SEQ ID NO: 31 - RNA, 21 nt, Artificial Sequence
  siRNA
  modified_base 2: /mod_base="OTHER" /note="2'-fluoro deoxyuridine"
  modified_base 8: /mod_base="OTHER" /note="2'-fluoro deoxyuridine"
  modified_base 20: /mod_base="OTHER" /note="deoxy-thymidine"
  modified_base 21: /mod_base="OTHER" /note="deoxy-thymidine"
gngagaangaguacuuuaann

SEQ ID NO: 32 - RNA, 21 nt, Artificial Sequence
  siRNA
  modified_base 20: /mod_base="OTHER" /note="deoxy-thymidine"
  modified_base 21: /mod_base="OTHER" /note="deoxy-thymidine"
uuaaaguacucauucucacnn

SEQ ID NO: 33 - RNA, 21 nt, Artificial Sequence
  siRNA
  modified_base 1: /mod_base="gm"
  modified_base 2: /mod_base="um"
  modified_base 18: /mod_base="OTHER" /note="2'-O-methyl-adenosine"
  modified_base 19: /mod_base="OTHER" /note="2'-O-methyl-adenosine"
  modified_base 20: /mod_base="OTHER" /note="deoxy-thymidine"
  modified_base 21: /mod_base="OTHER" /note="deoxy-thymidine"
gngagaaugaguacuuuaann

SEQ ID NO: 34 - RNA, 21 nt, Artificial Sequence
  siRNA
  modified_base 20: /mod_base="OTHER" /note="deoxy-thymidine"
  modified_base 21: /mod_base="OTHER" /note="deoxy-thymidine"
uuaaaguacucauucucacnn

SEQ ID NO: 35 - RNA, 21 nt, Artificial Sequence
  siRNA
  modified_base 4: /mod_base="OTHER" /note="2'-O-methyl-adenosine"
  modified_base 6: /mod_base="OTHER" /note="2'-O-methyl-adenosine"
  modified_base 7: /mod_base="OTHER" /note="2'-O-methyl-adenosine"
  modified_base 10: /mod_base="OTHER" /note="2'-O-methyl-adenosine"
  modified_base 13: /mod_base="OTHER" /note="2'-O-methyl-adenosine"
  modified_base 18: /mod_base="OTHER" /note="2'-O-methyl-adenosine"
  modified_base 19: /mod_base="OTHER" /note="2'-O-methyl-adenosine"
  modified_base 20: /mod_base="OTHER" /note="deoxy-thymidine"
  modified_base 21: /mod_base="OTHER" /note="deoxy-thymidine"
gugagaaugaguacuuuaann

SEQ ID NO: 36 - RNA, 21 nt, Artificial Sequence
  siRNA
  modified_base 20: /mod_base="OTHER" /note="deoxy-thymidine"
  modified_base 21: /mod_base="OTHER" /note="deoxy-thymidine"
uuaaaguacucauucucacnn

SEQ ID NO: 37 - RNA, 21 nt, Artificial Sequence
  siRNA
  modified_base 4: /mod_base="OTHER" /note="2'-fluoro deoxyadenosine"
  modified_base 6: /mod_base="OTHER" /note="2'-fluoro deoxyadenosine"
  modified_base 7: /mod_base="OTHER" /note="2'-fluoro deoxyadenosine"
  modified_base 10: /mod_base="OTHER" /note="2'-fluoro deoxyadenosine"
  modified_base 13: /mod_base="OTHER" /note="2'-fluoro deoxyadenosine"
  modified_base 18: /mod_base="OTHER" /note="2'-fluoro deoxyadenosine"
  modified_base 19: /mod_base="OTHER" /note="2'-fluoro deoxyadenosine"
  modified_base 20: /mod_base="OTHER" /note="deoxy-thymidine"
  modified_base 21: /mod_base="OTHER" /note="deoxy-thymidine"
gugagaaugaguacuuuaann

SEQ ID NO: 38 - RNA, 21 nt, Artificial Sequence
  siRNA
  modified_base 20: /mod_base="OTHER" /note="deoxy-thymidine"
  modified_base 21: /mod_base="OTHER" /note="deoxy-thymidine"
uuaaaguacucauucucacnn

SEQ ID NO: 39 - RNA, 21 nt, Artificial Sequence
  siRNA
  modified_base 2: /mod_base="um"
  modified_base 8: /mod_base="um"
  modified_base 12: /mod_base="um"
  modified_base 16: /mod_base="um"
  modified_base 20: /mod_base="OTHER" /note="deoxy-thymidine"
  modified_base 21: /mod_base="OTHER" /note="deoxy-thymidine"
gngagaangagnacunuaann

SEQ ID NO: 40 - RNA, 21 nt, Artificial Sequence
  siRNA
  modified_base 5: /mod_base="gm"
  modified_base 16: /mod_base="um"
  modified_base 20: /mod_base="OTHER" /note="deoxy-thymidine"
  modified_base 21: /mod_base="OTHER" /note="deoxy-thymidine"
uuaagguacucauucncacnn

SEQ ID NO: 41 - RNA, 21 nt, Artificial Sequence
  siRNA
  modified_base 2: /mod_base="OTHER" /note="2'-fluoro deoxyuridine"
  modified_base 4: /mod_base="OTHER" /note="2'-fluoro deoxyadenosine"
  modified_base 6: /mod_base="OTHER" /note="2'-fluoro deoxyadenosine"
  modified_base 7: /mod_base="OTHER" /note="2'-fluoro deoxyadenosine"
  modified_base 8: /mod_base="OTHER" /note="2'-fluoro deoxyuridine"
  modified_base 20: /mod_base="OTHER" /note="deoxy-thymidine"
  modified_base 21: /mod_base="OTHER" /note="deoxy-thymidine"
gngagaangaguacuuuaann

SEQ ID NO: 42 - RNA, 21 nt, Artificial Sequence
  siRNA
  modified_base 20: /mod_base="OTHER" /note="deoxy-thymidine"
  modified_base 21: /mod_base="OTHER" /note="deoxy-thymidine"
uuaaaguacucauucucacnn

SEQ ID NO: 43 - RNA, 21 nt, Artificial Sequence
  siRNA
  modified_base 20: /mod_base="OTHER" /note="deoxy-thymidine"
  modified_base 21: /mod_base="OTHER" /note="deoxy-thymidine"
gugagaaugaguacuuuaann

SEQ ID NO: 44 - RNA, 21 nt, Artificial Sequence
  siRNA
  modified_base 1: /mod_base="OTHER" /note="2'-fluoro deoxyuridine"
  modified_base 3: /mod_base="OTHER" /note="2'-fluoro deoxyadenosine"
  modified_base 5: /mod_base="OTHER" /note="2'-fluoro deoxyadenosine"
  modified_base 7: /mod_base="OTHER" /note="2'-fluoro deoxyuridine"
  modified_base 8: /mod_base="OTHER" /note="2'-fluoro deoxyadenosine"
  modified_base 20: /mod_base="OTHER" /note="deoxy-thymidine"
  modified_base 21: /mod_base="OTHER" /note="deoxy-thymidine"
nuaaagnacucauucucacnn

SEQ ID NO: 45 - RNA, 21 nt, Artificial Sequence
  siRNA
  modified_base 2: /mod_base="um"
  modified_base 4: /mod_base="OTHER" /note="2'-O-methyl-adenosine"
  modified_base 6: /mod_base="OTHER" /note="2'-O-methyl-adenosine"
  modified_base 7: /mod_base="OTHER" /note="2'-O-methyl-adenosine"
  modified_base 8: /mod_base="um"
  modified_base 20: /mod_base="OTHER" /note="deoxy-thymidine"
  modified_base 21: /mod_base="OTHER" /note="deoxy-thymidine"
gngagaangaguacuuuaann

SEQ ID NO: 46 - RNA, 21 nt, Artificial Sequence
  siRNA
  modified_base 20: /mod_base="OTHER" /note="deoxy-thymidine"
  modified_base 21: /mod_base="OTHER" /note="deoxy-thymidine"
uuaaaguacucauucucacnn

SEQ ID NO: 47 - RNA, 21 nt, Artificial Sequence
  siRNA
  modified_base 2: /mod_base="um"
  modified_base 4: /mod_base="OTHER" /note="2'-O-methyl-adenosine"
  modified_base 6: /mod_base="OTHER" /note="2'-O-methyl-adenosine"
  modified_base 7: /mod_base="OTHER" /note="2'-O-methyl-adenosine"
  modified_base 8: /mod_base="um"
  modified_base 20: /mod_base="OTHER" /note="deoxy-thymidine"
  modified_base 21: /mod_base="OTHER" /note="deoxy-thymidine"
gngagaangaguacuuuaann

SEQ ID NO: 48 - RNA, 21 nt, Artificial Sequence
  siRNA
  modified_base 13: /mod_base="OTHER" /note="2'-fluoro deoxyuridine"
  modified_base 15: /mod_base="OTHER" /note="2'-fluoro deoxycytosine"
  modified_base 17: /mod_base="OTHER" /note="2'-fluoro deoxycytosine"
  modified_base 19: /mod_base="OTHER" /note="2'-fluoro deoxycytosine"
  modified_base 20: /mod_base="OTHER" /note="deoxy-thymidine"
  modified_base 21: /mod_base="OTHER" /note="deoxy-thymidine"
uuaaaguacucanucucacnn

SEQ ID NO: 49 - RNA, 21 nt, Artificial Sequence
  siRNA
  modified_base 2: /mod_base="OTHER" /note="2'-fluoro deoxyuridine"
  modified_base 4: /mod_base="OTHER" /note="2'-fluoro deoxyadenosine"
  modified_base 6: /mod_base="OTHER" /note="2'-fluoro deoxyadenosine"
  modified_base 7: /mod_base="OTHER" /note="2'-fluoro deoxyadenosine"
  modified_base 8: /mod_base="OTHER" /note="2'-fluoro deoxyuridine"
  modified_base 20: /mod_base="OTHER" /note="deoxy-thymidine"
  modified_base 21: /mod_base="OTHER" /note="deoxy-thymidine"
gngagaangaguacuuuaann

SEQ ID NO: 50 - RNA, 21 nt, Artificial Sequence
  siRNA
  modified_base 12: /mod_base="OTHER" /note="2'-O-methyl-adenosine"
  modified_base 14: /mod_base="um"
  modified_base 16: /mod_base="um"
  modified_base 18: /mod_base="OTHER" /note="2'-O-methyl-adenosine"
  modified_base 20: /mod_base="OTHER" /note="deoxy-thymidine"
  modified_base 21: /mod_base="OTHER" /note="deoxy-thymidine"
uuaaaguacucauncncacnn

SEQ ID NO: 51 - RNA, 21 nt, Artificial Sequence
  siRNA
  modified_base 1: /mod_base="gm"
  modified_base 3: /mod_base="gm"
  modified_base 5: /mod_base="gm"
  modified_base 9: /mod_base="gm"
  modified_base 11: /mod_base="gm"
  modified_base 20: /mod_base="OTHER" /note="deoxy-thymidine"
  modified_base 21: /mod_base="OTHER" /note="deoxy-thymidine"
gugagaaugaguacuuuaann

SEQ ID NO: 52 - RNA, 21 nt, Artificial Sequence
  siRNA
  modified_base 20: /mod_base="OTHER" /note="deoxy-thymidine"
  modified_base 21: /mod_base="OTHER" /note="deoxy-thymidine"
uuaaaguacucauucucacnn

SEQ ID NO: 53 - RNA, 21 nt, Artificial Sequence
  siRNA
  modified_base 2: /mod_base="um"
  modified_base 8: /mod_base="um"
  modified_base 12: /mod_base="um"
  modified_base 15: /mod_base="um"
  modified_base 16: /mod_base="um"
  modified_base 17: /mod_base="um"
  modified_base 20: /mod_base="OTHER" /note="deoxy-thymidine"
  modified_base 21: /mod_base="OTHER" /note="deoxy-thymidine"
gngagaangagnacnnnaann

SEQ ID NO: 54 - RNA, 21 nt, Artificial Sequence
  siRNA
  modified_base 20: /mod_base="OTHER" /note="deoxy-thymidine"
  modified_base 21: /mod_base="OTHER" /note="deoxy-thymidine"
uuaaaguacucauucucacnn

SEQ ID NO: 55 - RNA, 21 nt, Artificial Sequence
  siRNA
  modified_base 4: /mod_base="OTHER" /note="2'-O-methyl-adenosine"
  modified_base 10: /mod_base="OTHER" /note="2'-O-methyl-adenosine"
  modified_base 13: /mod_base="OTHER" /note="2'-O-methyl-adenosine"
  modified_base 18: /mod_base="OTHER" /note="2'-O-methyl-adenosine"
  modified_base 20: /mod_base="OTHER" /note="deoxy-thymidine"
  modified_base 21: /mod_base="OTHER" /note="deoxy-thymidine"
gugagaaugaguacuuuaann

SEQ ID NO: 56 - RNA, 21 nt, Artificial Sequence
  siRNA
  modified_base 1: /mod_base="um"
  modified_base 14: /mod_base="um"
  modified_base 20: /mod_base="OTHER" /note="deoxy-thymidine"
  modified_base 21: /mod_base="OTHER" /note="deoxy-thymidine"
nuaaaguacucauncucacnn

SEQ ID NO: 57 - RNA, 21 nt, Artificial Sequence
  siRNA
  modified_base 3: /mod_base="gm"
  modified_base 5: /mod_base="gm"
  modified_base 9: /mod_base="gm"
  modified_base 11: /mod_base="gm"
  modified_base 20: /mod_base="OTHER" /note="deoxy-thymidine"
  modified_base 21: /mod_base="OTHER" /note="deoxy-thymidine"
gugagaaugaguacuuuaann

SEQ ID NO: 58 - RNA, 21 nt, Artificial Sequence
  siRNA
  modified_base 7: /mod_base="um"
  modified_base 16: /mod_base="um"
  modified_base 20: /mod_base="OTHER" /note="deoxy-thymidine"
  modified_base 21: /mod_base="OTHER" /note="deoxy-thymidine"
uuaaagnacucauucncacnn

SEQ ID NO: 59 - RNA, 21 nt, Artificial Sequence
  siRNA
guacugguccguuagcaaauu

SEQ ID NO: 60 - RNA, 21 nt, Artificial Sequence
  siRNA
uuugcuaacggaccaguacuu

SEQ ID NO: 61 - RNA, 19 nt, Artificial Sequence
  siRNA
ggaacaaaugcgucccaua

SEQ ID NO: 62 - RNA, 19 nt, Artificial Sequence
  siRNA
auacaaacuccguaccuua

SEQ ID NO: 63 - RNA, 19 nt, Artificial Sequence
  siRNA
uaugagaaccugcacacua

SEQ ID NO: 64 - RNA, 19 nt, Artificial Sequence
  siRNA
gcuccgaucccacuaguga

SEQ ID NO: 65 - RNA, 19 nt, Artificial Sequence
  siRNA
gaacaucacgggcaauuaa

SEQ ID NO: 66 - RNA, 19 nt, Artificial Sequence
  siRNA
gaagcacaguaccgauuua

SEQ ID NO: 67 - RNA, 19 nt, Artificial Sequence
  siRNA
ggagaugguuucacccaaa

SEQ ID NO: 68 - RNA, 19 nt, Artificial Sequence
  siRNA
ggacguucauugugauuga